European Patent Specification EP 3 903 107 B1, published January 29, 2025. Title: Method for detecting the presence and quantity of receptor LRP8 and its proteolitic fragments, diagnostic kit and related antibodies. Applicant: RUSSO, Claudio. The sequence listing filed with the application follows.

SEQUENCE LISTING (82 sequences)

SEQ ID NO: 1 - protein, 127 aa, Homo sapiens
IALLCMSGYLIWRNWKRKNTKSMNFDNPVYRKTTEEEDEDELHIGRTAQIGHVYPAAISSFDRPLWAEPCLGETREPEDPAPALKELFVLPGEPRSQLHQLPKNPLSELPVVKSKRVALSLEDDGLP

SEQ ID NO: 2 - protein, 21 aa, Homo sapiens
IALLCMSGYLIWRNWKRKNTK

SEQ ID NO: 3 - protein, 15 aa, Homo sapiens
NWKRKNTKSMNFDNP

SEQ ID NO: 4 - protein, 16 aa, Homo sapiens
NPVYRKTTEEEDEDEL

SEQ ID NO: 5 - protein, 14 aa, Homo sapiens
DEDELHIGRTAQIG

SEQ ID NO: 6 - protein, 17 aa, Homo sapiens
RTAQIGHVYPAAISSFD

SEQ ID NO: 7 - protein, 20 aa, Homo sapiens
DRPLWAEPCLGETREPEDPA

SEQ ID NO: 8 - protein, 26 aa, Homo sapiens
DPAPALKELFVLPGEPRSQLHQLPKN

SEQ ID NO: 9 - protein, 24 aa, Homo sapiens
NPLSELPVVKSKRVALSLEDDGLP

SEQ ID NO: 10 - protein, 21 aa, Homo sapiens
VIGIIVPIVVIALLCMSGYLI

SEQ ID NO: 11 - protein, 4 aa, Homo sapiens
VVIA

SEQ ID NO: 12 - protein, 5 aa, Homo sapiens
DNPVY

SEQ ID NO: 13 - protein, 59 aa, Homo sapiens
AISSFDRPLWAEPCLGETREPEDPAPALKELFVLPGEPRSQLHQLPKNPLSELPVVKSK

SEQ ID NO: 14 - protein, 963 aa, Homo sapiens
MGLPEPGPLRLLALLLLLLLLLLLQLQHLAAAAADPLLGGQGPAKDCEKDQFQCRNERCIPSVWRCDEDDDCLDHSDEDDCPKKTCADSDFTCDNGHCIHERWKCDGEEECPDGSDESEATCTKQVCPAEKLSCGPTSHKCVPASWRCDGEKDCEGGADEAGCATLCAPHEFQCGNRSCLAAVFVCDGDDDCGDGSDERGCADPACGPREFRCGGDGGGACIPERWVCDRQFDCEDRSDEAAELCGRPGPGATSAPAACATASQFACRSGECVHLGWRCDGDRDCKDKSDEADCPLGTCRGDEFQCGDGTCVLAIKHCNQEQDCPDGSDEAGCLQGLNECLHNNGGCSHICTDLKIGFECTCPAGFQLLDQKTCGDIDECKDPDACSQICVNYKGYFKCECYPGYEMDLLTKNCKAAAGKSPSLIFTNRHEVRRIDLVKRNYSRLIPMLKNVVALDVEVATNRIYWCDLSYRKIYSAYMDKASDPKEQEVLIDEQLHSPEGLAVDWVHKHIYWTDSGNKTISVATVDGGRRRTLFSRNLSEPRAIAVDPLRGFMYWSDWGDQAKIEKSGLNGVDRQTLVSDNIEWPNGITLDLLSQRLYWVDSKLHQLSSIDFSGGNRKTLISSTDFLSHPFGIAVFEDKVFWTDLENEAIFSANRLNGLEISILAENLNNPHDIVIFHELKQPRAPDACELSVQPNGGCEYLCLPAPQISSHSPKYTCACPDTMWLGPDMKRCYRAPQSTSTTTLASTMTRTVPATTRAPGTTVHRSTYQNHSTETPSLTAAVPSSVSVPRAPSISPSTLSPATSNHSQHYANEDSKMGSTVTAAVIGIIVPIVVIALLCMSGYLIWRNWKRKNTKSMNFDNPVYRKTTEEEDEDELHIGRTAQIGHVYPAAISSFDRPLWAEPCLGETREPEDPAPALKELFVLPGEPRSQLHQLPKNPLSELPVVKSKRVALSLEDDGLP

SEQ ID NO: 15 - protein, 183 aa, Homo sapiens
TAAVPSSVSVPRAPSISPSTLSPATSNHSQHYANEDSKMGSTVTAAVIGIIVPIVVIALLCMSGYLIWRNWKRKNTKSMNFDNPVYRKTTEEEDEDELHIGRTAQIGHVYPAAISSFDRPLWAEPCLGETREPEDPAPALKELFVLPGEPRSQLHQLPKNPLSELPVVKSKRVALSLEDDGLP

SEQ ID NO: 16 - protein, 91 aa, Homo sapiens
NEDSKMGSTVTAAVIGIIVPIVVIALLCMSGYLIWRNWKRKNTKSMNFDNPVYRKTTEEEDEDELHIGRTAQIGHVYPARVALSLEDDGLP

SEQ ID NO: 17 - protein, 124 aa, Homo sapiens
TAAVPSSVSVPRAPSISPSTLSPATSNHSQHYANEDSKMGSTVTAAVIGIIVPIVVIALLCMSGYLIWRNWKRKNTKSMNFDNPVYRKTTEEEDEDELHIGRTAQIGHVYPARVALSLEDDGLP

SEQ ID NO: 18 - protein, 183 aa, Homo sapiens; identical to SEQ ID NO: 15

SEQ ID NO: 19 - DNA, 57 bp, Homo sapiens
atgggatggagctggatctttctcttcctcctgtcaggaactgcaggtgtccactct

SEQ ID NO: 20 - DNA, 90 bp, Homo sapiens
gaggtccagctgcaacagtctggacctgtgctggtgaagcctggggcttcagtgaagatgtcctgtaaggcttctggatacaaattcact

SEQ ID NO: 21 - DNA, 15 bp, Homo sapiens
gactactttatgaac

SEQ ID NO: 22 - DNA, 42 bp, Homo sapiens
tgggtgaagaagagccatggaaagagccttgagtggattgga

SEQ ID NO: 23 - DNA, 51 bp, Homo sapiens
gttattaatccttacaacggtggtactagatacaaccagaagttcaagggc

SEQ ID NO: 24 - DNA, 96 bp, Homo sapiens
aaggccacattgactgttgacaagtcctccagcacagcctacatggagctcaacagcctgacatttgaggactctgcagtctattactgtgcaagg

SEQ ID NO: 25 - DNA, 30 bp, Homo sapiens
gagacggtagaccttgcctggtttgttcac

SEQ ID NO: 26 - DNA, 33 bp, Homo sapiens
tggggccaagggactctggtcactgtctctgca

SEQ ID NO: 27 - protein, 19 aa, Homo sapiens
MGWSWIFLFLLSGTAGVHS

SEQ ID NO: 28 - protein, 30 aa, Homo sapiens
EVQLQQSGPVLVKPGASVKMSCKASGYKFT

SEQ ID NO: 29 - protein, 5 aa, Homo sapiens
DYFMN

SEQ ID NO: 30 - protein, 14 aa, Homo sapiens
WVKKSHGKSLEWIG

SEQ ID NO: 31 - protein, 17 aa, Homo sapiens
VINPYNGGTRYNQKFKG

SEQ ID NO: 32 - protein, 32 aa, Homo sapiens
KATLTVDKSSSTAYMELNSLTFEDSAVYYCAR

SEQ ID NO: 33 - protein, 10 aa, Homo sapiens
ETVDLAWFVH

SEQ ID NO: 34 - protein, 11 aa, Homo sapiens
WGQGTLVTVSA

SEQ ID NO: 35 - DNA, 57 bp, Homo sapiens
atgaagttgcctgttaggctgttggtgctgatgttctggattcctgcttccagcagt

SEQ ID NO: 36 - DNA, 69 bp, Homo sapiens
gatgttttgatgacccaaactccaccctccctgcctgtcactcttggagatcaggcctccatctcttgc

SEQ ID NO: 37 - DNA, 48 bp, Homo sapiens
agatctagtcagagtattgtatatagtaatggaaacacctacttagaa

SEQ ID NO: 38 - DNA, 45 bp, Homo sapiens
tggtacctgcagaagccaggccagtctccaaagctcctgatctac

SEQ ID NO: 39 - DNA, 21 bp, Homo sapiens
aaagtttccaaccgattttct

SEQ ID NO: 40 - DNA, 96 bp, Homo sapiens
ggggtcccagacaggttcagtggcagtggatcagggacagatttcacactcaagatcagcagagtggaggctgaggatctgggaatttattactgc

SEQ ID NO: 41 - DNA, 27 bp, Homo sapiens
tttcaaggttcacatgttccgctcacg

SEQ ID NO: 42 - DNA, 30 bp, Homo sapiens
ttcggtgctgggaccaagctggagctgaaa

SEQ ID NO: 43 - protein, 19 aa, Homo sapiens
MKLPVRLLVLMFWIPASSS

SEQ ID NO: 44 - protein, 23 aa, Homo sapiens
DVLMTQTPPSLPVTLGDQASISC

SEQ ID NO: 45 - protein, 16 aa, Homo sapiens
RSSQSIVYSNGNTYLE

SEQ ID NO: 46 - protein, 15 aa, Homo sapiens
WYLQKPGQSPKLLIY

SEQ ID NO: 47 - protein, 7 aa, Homo sapiens
KVSNRFS

SEQ ID NO: 48 - protein, 32 aa, Homo sapiens
GVPDRFSGSGSGTDFTLKISRVEAEDLGIYYC

SEQ ID NO: 49 - protein, 9 aa, Homo sapiens
FQGSHVPLT

SEQ ID NO: 50 - protein, 10 aa, Homo sapiens
FGAGTKLELK

SEQ ID NO: 51 - DNA, 57 bp, Homo sapiens; identical to SEQ ID NO: 19

SEQ ID NO: 52 - DNA, 90 bp, Homo sapiens; identical to SEQ ID NO: 20

SEQ ID NO: 53 - DNA, 15 bp, Homo sapiens
gaccactttatgaac

SEQ ID NO: 54 - DNA, 42 bp, Homo sapiens
tgggtgaagaagaaccatggaaagagccttgagtggattggg

SEQ ID NO: 55 - DNA, 51 bp, Homo sapiens
gttattaatccttacaacggtggtactaggctcaacccgaagtttaagggc

SEQ ID NO: 56 - DNA, 96 bp, Homo sapiens
aaggccacattgactgttgacaagtcctccagcacagtctacatggagctcaacagcctgacatttgaggactctgcagtctattactgtgcaagg

SEQ ID NO: 57 - DNA, 30 bp, Homo sapiens
gagactatagaccttgcctggtttgcttat

SEQ ID NO: 58 - DNA, 33 bp, Homo sapiens
tggggccaggggactctggtcactgtctctgca

SEQ ID NO: 59 - protein, 19 aa, Homo sapiens
MGWSWIFLFLLSGTAGVHS

SEQ ID NO: 60 - protein, 30 aa, Homo sapiens; identical to SEQ ID NO: 28

SEQ ID NO: 61 - protein, 5 aa, Homo sapiens
DHFMN

SEQ ID NO: 62 - protein, 14 aa, Homo sapiens
WVKKNHGKSLEWIG

SEQ ID NO: 63 - protein, 17 aa, Homo sapiens
VINPYNGGTRLNPKFKG

SEQ ID NO: 64 - protein, 32 aa, Homo sapiens
KATLTVDKSSSTVYMELNSLTFEDSAVYYCAR

SEQ ID NO: 65 - protein, 10 aa, Homo sapiens
ETIDLAWFAY

SEQ ID NO: 66 - protein, 11 aa, Homo sapiens
WGQGTLVTVSA

SEQ ID NO: 67 - DNA, 57 bp, Homo sapiens
atgaagttgcctgttaggctgttggtgctgatgttctggattcctgctaccagcagt

SEQ ID NO: 68 - DNA, 69 bp, Homo sapiens
gatgttttgatgactcaaactccaccctccctgcctgtcactcttggagatcaggcctccatctcttgc

SEQ ID NO: 69 - DNA, 48 bp, Homo sapiens
agatctagtcagagtattgtatatagtaatggaaaaacctatttagaa

SEQ ID NO: 70 - DNA, 45 bp, Homo sapiens
tggtacctgcagaagccaggccagtctccaaagctcctgatgtac

SEQ ID NO: 71 - DNA, 21 bp, Homo sapiens
aaagtttccaaccgattttct

SEQ ID NO: 72 - DNA, 96 bp, Homo sapiens
ggggtcccagacaggttcagtggcagtggatcagggacagatttcacactcaagatcagcagcgtggaggctgaggatctgggaatttattactgc

SEQ ID NO: 73 - DNA, 27 bp, Homo sapiens
tttcaaggttcacatgttccgctcacg

SEQ ID NO: 74 - DNA, 30 bp, Homo sapiens; identical to SEQ ID NO: 42

SEQ ID NO: 75 - protein, 19 aa, Homo sapiens
MKLPVRLLVLMFWIPATSS

SEQ ID NO: 76 - protein, 23 aa, Homo sapiens
DVLMTQTPPSLPVTLGDQASISC

SEQ ID NO: 77 - protein, 16 aa, Homo sapiens
RSSQSIVYSNGKTYLE

SEQ ID NO: 78 - protein, 15 aa, Homo sapiens
WYLQKPGQSPKLLMY

SEQ ID NO: 79 - protein, 7 aa, Homo sapiens
KVSNRFS

SEQ ID NO: 80 - protein, 32 aa, Homo sapiens
GVPDRFSGSGSGTDFTLKISSVEAEDLGIYYC

SEQ ID NO: 81 - protein, 9 aa, Homo sapiens
FQGSHVPLT

SEQ ID NO: 82 - protein, 10 aa, Homo sapiens
FGAGTKLELK